European Patent Application EP 4 194 488 A1, published June 14, 2023. Title: POLYPEPTIDE, PHOTORESIST COMPOSITION INCLUDING THE SAME, AND METHOD OF FORMING PATTERN USING THE SAME. Applicant: Samsung Electronics Co., Ltd. The sequence listing filed with the application follows.

SEQUENCE LISTING (20 sequences)

SEQ ID NO: 1 - protein, 6 aa, Artificial Sequence
  Artificial polypeptide
  FirstRepeatUnit1 (1)..(6)
GAGAGS

SEQ ID NO: 2 - protein, 4 aa, Artificial Sequence
  Artificial polypeptide
  FirstRepeatUnit2 (1)..(4)
GAAS

SEQ ID NO: 3 - protein, 4 aa, Artificial Sequence
  Artificial polypeptide
  SecondRepeatUnit1 (1)..(4)
GAGY

SEQ ID NO: 4 - protein, 6 aa, Artificial Sequence
  Artificial polypeptide
  SecondRepeatUnit2 (1)..(6)
GAGAGY

SEQ ID NO: 5 - protein, 8 aa, Artificial Sequence
  Artificial polypeptide
  SecondRepeatUnit3 (1)..(8)
GAGVGAGY

SEQ ID NO: 6 - protein, 8 aa, Artificial Sequence
  Artificial polypeptide
  SecondRepeatUnit4 (1)..(8)
GAGAGAGY

SEQ ID NO: 7 - protein, 6 aa, Artificial Sequence
  Artificial polypeptide
  ThirdRepeatUnit1 (1)..(6)
DEDEDE

SEQ ID NO: 8 - protein, 6 aa, Artificial Sequence
  Artificial polypeptide
  ThirdRepeatUnit2 (1)..(6)
DDDDDD

SEQ ID NO: 9 - protein, 4 aa, Artificial Sequence
  Artificial polypeptide
  RegionH1 (1)..(4)
GAAS

SEQ ID NO: 10 - protein, 10 aa, Artificial Sequence
  Artificial polypeptide
  RegionH2 (1)..(10)
GAGAGSGAAS

SEQ ID NO: 11 - protein, 84 aa, Artificial Sequence
  Artificial polypeptide
  SynthesisExample1 (1)..(84): HA8B4
GAGAGSGAASGAGAGSGAGAGSGAGAGSGAGAGSGAGAGSGAGAGSGAGAGSGAGAGSGAGAGYGAGVGAGYGAGYGAGAGAGY

SEQ ID NO: 12 - protein, 86 aa, Artificial Sequence
  Artificial polypeptide
  SynthesisExample2 (1)..(86): HA8B4D2
GAGAGSGAASGAGAGSGAGAGSGAGAGSGAGAGSGAGAGSGAGAGSGAGAGSGAGAGSGAGAGYGAGVGAGYGAGYGAGAGAGYDD

SEQ ID NO: 13 - protein, 90 aa, Artificial Sequence
  Artificial polypeptide
  SynthesisExample3 (1)..(90): HA8B4D6
GAGAGSGAASGAGAGSGAGAGSGAGAGSGAGAGSGAGAGSGAGAGSGAGAGSGAGAGSGAGAGYGAGVGAGYGAGYGAGAGAGYDDDDDD

SEQ ID NO: 14 - protein, 86 aa, Artificial Sequence
  Artificial polypeptide
  SynthesisExample4 (1)..(86): HA8B4E2
GAGAGSGAASGAGAGSGAGAGSGAGAGSGAGAGSGAGAGSGAGAGSGAGAGSGAGAGSGAGAGYGAGVGAGYGAGYGAGAGAGYEE

SEQ ID NO: 15 - protein, 86 aa, Artificial Sequence
  Artificial polypeptide
  SynthesisExample5 (1)..(86): HA8B4DE
GAGAGSGAASGAGAGSGAGAGSGAGAGSGAGAGSGAGAGSGAGAGSGAGAGSGAGAGSGAGAGYGAGVGAGYGAGYGAGAGAGYDE

SEQ ID NO: 16 - protein, 90 aa, Artificial Sequence
  Artificial polypeptide
  SynthesisExample6 (1)..(90): HA8B4(DE)3
GAGAGSGAASGAGAGSGAGAGSGAGAGSGAGAGSGAGAGSGAGAGSGAGAGSGAGAGSGAGAGYGAGVGAGYGAGYGAGAGAGYDEDEDE

SEQ ID NO: 17 - protein, 42 aa, Artificial Sequence
  Artificial polypeptide
  SynthesisExample7 (1)..(42): HA1B4
GAGAGSGAASGAGAGSGAGAGYGAGVGAGYGAGYGAGAGAGY

SEQ ID NO: 18 - protein, 56 aa, Artificial Sequence
  Artificial polypeptide
  SynthesisExample8 (1)..(56): HA1B6
GAGAGSGAASGAGAGSGAGAGYGAGVGAGYGAGAGYGAGVGAGYGAGYGAGAGAGY

SEQ ID NO: 19 - protein, 48 aa, Artificial Sequence
  Artificial polypeptide
  SynthesisExample9 (1)..(48): HA1B4D6
GAGAGSGAASGAGAGSGAGAGYGAGVGAGYGAGYGAGAGAGYDDDDDD

SEQ ID NO: 20 - protein, 62 aa, Artificial Sequence
  Artificial polypeptide
  SynthesisExample10 (1)..(62): HA1B6D6
GAGAGSGAASGAGAGSGAGAGYGAGVGAGYGAGAGYGAGVGAGYGAGYGAGAGAGYDDDDDD